European Patent Application EP 4 174 085 A1, published May 3, 2023. Title: Anti-SARS-CoV-2 antibody and method of detecting SARS-CoV-2 using said antibody and kit comprising said antibody. Applicant: Kanto Kagaku Kabushiki Kaisha. The sequence listing filed with the application follows.

SEQUENCE LISTING (15 sequences)

SEQ ID NO: 1 - protein, 419 aa, Human coronavirus
MSDNGPQNQRNAPRITFGGPSDSTGSNQNGERSGARSKQRRPQGLPNNTASWFTALTQHGKEDLKFPRGQGVPINTNSSPDDQIGYYRRATRRIRGGDGKMKDLSPRWYFYYLGTGPEAGLPYGANKDGIIWVATEGALNTPKDHIGTRNPANNAAIVLQLPQGTTLPKGFYAEGSRGGSQASSRSSSRSRNSSRNSTPGSSRGTSPARMAGNGGDAALALLLLDRLNQLESKMSGKGQQQQGQTVTKKSAAEASKKPRQKRTATKAYNVTQAFGRRGPEQTQGNFGDQELIRQGTDYKHWPQIAQFAPSASAFFGMSRIGMEVTPSGTWLTYTGAIKLDDKDPNFKDQVILLNKHIDAYKTFPPTEPKKDKKKKADETQALPQRQKKQQTVTLLPAADLDDFSKQLQQSMSSADSTQA

SEQ ID NO: 2 - protein, 299 aa, Human coronavirus
LPYGANKDGIIWVATEGALNTPKDHIGTRNPANNAAIVLQLPQGTTLPKGFYAEGSRGGSQASSRSSSRSRNSSRNSTPGSSRGTSPARMAGNGGDAALALLLLDRLNQLESKMSGKGQQQQGQTVTKKSAAEASKKPRQKRTATKAYNVTQAFGRRGPEQTQGNFGDQELIRQGTDYKHWPQIAQFAPSASAFFGMSRIGMEVTPSGTWLTYTGAIKLDDKDPNFKDQVILLNKHIDAYKTFPPTEPKKDKKKKADETQALPQRQKKQQTVTLLPAADLDDFSKQLQQSMSSADSTQA

SEQ ID NO: 3 - RNA, 1260 nt, Human coronavirus
auguccgacaaugggccccagaaucagcgaaaugcgccuaggauuaccuuuggcggacccagcgacagcacaggcagcaaccagaauggcgagagaaguggcgcucgcucuaagcagcgccgcccucaagggcucccgaauaacaccgccuccugguucacugcacucacgcagcaugggaaggaggaucugaaauuccccagaggucaagguguuccuaucaacaccaacuccucacccgacgaucagaucggcuauuauaggcgggcuacaagacggauacggggcggugacgggaaaaugaaagaucugagcccacggugguacuucuacuaucucgguacugguccugaggcaggacugccauauggggcaaacaaagaugggaucauuuggguggcuaccgaaggugccuugaacaccccaaaggaccacauaggcacgagaaaccccgccaauaaugcugcaaucguccugcaacugccacaaggaacaacucuccccaaaggguucuacgcagaagggucacgaggcggaucucaagccucaaguaggagcucuuccaggagucgaaauagcucccggaacucaacacccggaagcucuagaggcaccagcccugcucgcauggccggaaauggcggagaugcagccuuggcacugcuucuucuggaccgccugaaccagcuggaaagcaagaugucagggaagggucagcagcagcagggccaaacugucaccaagaaaagugccgcagaggcuucaaagaagcccaggcagaaacggacugccaccaaagccuacaacgugacucaggcguuuggccguagagggccagaacagacgcagggaaacuuuggggaucaggaacuuaucaggcagggcacugacuacaaacauuggccccagauugcccaguuugcuccgucugcgucugcuuucuucggaaugucucguauuggcauggagguaacaccguccggaacauggcugaccuauacaggagccaucaaacuggaugacaaggacccuaacuuuaaggaccaagugauucuccugaauaagcacaucgaugccuacaaaaccuucccuccaacggagccuaagaaggacaagaagaagaaggccgaugagacucaagcccugccacagcgccagaagaaacaacagacagugaccuugcuuccagcugccgaucuggacgacuuuuccaaacagcugcagcagagcaugagcagugcggauuccacacaggcuuga

SEQ ID NO: 4 - DNA, 1260 bp, Human coronavirus
atgtccgacaatgggccccagaatcagcgaaatgcgcctaggattacctttggcggacccagcgacagcacaggcagcaaccagaatggcgagagaagtggcgctcgctctaagcagcgccgccctcaagggctcccgaataacaccgcctcctggttcactgcactcacgcagcatgggaaggaggatctgaaattccccagaggtcaaggtgttcctatcaacaccaactcctcacccgacgatcagatcggctattataggcgggctacaagacggatacggggcggtgacgggaaaatgaaagatctgagcccacggtggtacttctactatctcggtactggtcctgaggcaggactgccatatggggcaaacaaagatgggatcatttgggtggctaccgaaggtgccttgaacaccccaaaggaccacataggcacgagaaaccccgccaataatgctgcaatcgtcctgcaactgccacaaggaacaactctccccaaagggttctacgcagaagggtcacgaggcggatctcaagcctcaagtaggagctcttccaggagtcgaaatagctcccggaactcaacacccggaagctctagaggcaccagccctgctcgcatggccggaaatggcggagatgcagccttggcactgcttcttctggaccgcctgaaccagctggaaagcaagatgtcagggaagggtcagcagcagcagggccaaactgtcaccaagaaaagtgccgcagaggcttcaaagaagcccaggcagaaacggactgccaccaaagcctacaacgtgactcaggcgtttggccgtagagggccagaacagacgcagggaaactttggggatcaggaacttatcaggcagggcactgactacaaacattggccccagattgcccagtttgctccgtctgcgtctgctttcttcggaatgtctcgtattggcatggaggtaacaccgtccggaacatggctgacctatacaggagccatcaaactggatgacaaggaccctaactttaaggaccaagtgattctcctgaataagcacatcgatgcctacaaaaccttccctccaacggagcctaagaaggacaagaagaagaaggccgatgagactcaagccctgccacagcgccagaagaaacaacagacagtgaccttgcttccagctgccgatctggacgacttttccaaacagctgcagcagagcatgagcagtgcggattccacacaggcttga

SEQ ID NO: 5 - DNA, 33 bp, Artificial Sequence
  Forward primer
ggtggaggcggaagtctgccatatggggcaaac

SEQ ID NO: 6 - DNA, 33 bp, Artificial Sequence
  Reverse primer
caaaactagtgcggctcaagcctgtgtggaatc

SEQ ID NO: 7 - DNA, 20 bp, Artificial Sequence
  Forward primer
gccgcactagttttgtatag

SEQ ID NO: 8 - DNA, 33 bp, Artificial Sequence
  Reverse primer
acttccgcctccaccgtgatgatgatgatgatg

SEQ ID NO: 9 - DNA, 4553 bp, Artificial Sequence
  Vector
atttaggtgacactatagaactcacctatctccccaacacctaataacattcaatcactctttccactaaccacctatctacatcaccaatgggacatcatcatcatcatcacggtggaggcggaagtctgccatatggggcaaacaaagatgggatcatttgggtggctaccgaaggtgccttgaacaccccaaaggaccacataggcacgagaaaccccgccaataatgctgcaatcgtcctgcaactgccacaaggaacaactctccccaaagggttctacgcagaagggtcacgaggcggatctcaagcctcaagtaggagctcttccaggagtcgaaatagctcccggaactcaacacccggaagctctagaggcaccagccctgctcgcatggccggaaatggcggagatgcagccttggcactgcttcttctggaccgcctgaaccagctggaaagcaagatgtcagggaagggtcagcagcagcagggccaaactgtcaccaagaaaagtgccgcagaggcttcaaagaagcccaggcagaaacggactgccaccaaagcctacaacgtgactcaggcgtttggccgtagagggccagaacagacgcagggaaactttggggatcaggaacttatcaggcagggcactgactacaaacattggccccagattgcccagtttgctccgtctgcgtctgctttcttcggaatgtctcgtattggcatggaggtaacaccgtccggaacatggctgacctatacaggagccatcaaactggatgacaaggaccctaactttaaggaccaagtgattctcctgaataagcacatcgatgcctacaaaaccttccctccaacggagcctaagaaggacaagaagaagaaggccgatgagactcaagccctgccacagcgccagaagaaacaacagacagtgaccttgcttccagctgccgatctggacgacttttccaaacagctgcagcagagcatgagcagtgcggattccacacaggcttgatatagaatttacggctagcgccggatgcgacgccggtcgcgtcttatccggccttcctatatcaggctgtgtttaagacgccgccgcttcgcccaaatccctatgccggttcgacggctggacaaaatactgtttatcttcccagcgcaggcaggttaatgtaccaccccagcagcagccggtatccagcgcgtatataccttccggcgtacctttgccctccagcgatgcccagtgaccaaaggcgatgctgtattcttcagcgacagggccaggaatcgcaaaccacggtttcagtggggcaggggcctcttccggcgattcttactagctagtatgcataggtgctgaaatataaagtttgtgtttctaaaacacacgtggtacgtacgataacgtacagtgtttttccctccacttaaatcgaagggtagtgtcttggagcgcgcggagtaaacatatatggttcatatatgtccgtaggcacgtaaaaaaagcgagggattcgaattcccccggaacccccggttggggcccacgcctcgatcgagcaaaaaaaaaaaagaaaaaaaaaaaaaaagctttcccgcggccagcttggcgtaatcatggtcatagctgtttcctgtgtgaaattgttatccgctcacaattccacacaacatacgagccggaagcataaagtgtaaagcctggggtgcctaatgagtgagctaactcacattaattgcgttgcgctcactgcccgctttccagtcgggaaacctgtcgtgccggctgcattaatgaatcggccaacgcgcggggagaggcggtttgcgtattgggcgctcttccgcttcctcgctcactgactcgctgcgctcggtcgctcggctgcggcgagcggtatcagctcactcaaaggcggtaatacggttatccacagaatcaggggataacgcaggaaagaacatgtgagcaaaaggccagcaaaaggccaggaaccgtaaaaaggccgcgttgctggcgtttttccataggctccgcccccctgacgagcatcacaaaaatcgacgctcaagtcagaggtggcgaaacccgacaggactataaagataccaggcgtttccccctggaagctccctcgtgcgctctcctgttccgaccctgccgcttaccggatacctgtccgcctttctcccttcgggaagcgtggcgctttctcatagctcacgctgtaggtatctcagttcggtgtaggtcgttcgctccaagctgggctgtgtgcacgaaccccccgttcagcccgaccgctgcgccttatccggtaactatcgtcttgagtccaacccggtaagacacgacttatcgccactggcagcagccactggtaacaggattagcagagcgaggtatgtaggcggtgctacagagttcttgaagtggtggcctaactacggctacactagaagaacagtatttggtatctgcgctctgctgaagccagttaccttcggaaaaagagttggtagctcttgatccggcaaacaaaccaccgctggtagcggtggtttttttgcttgcaagcagcagattacgcgcagaaaaaaaggatctcaagaagatcctttgatcttttctacggggtctgacgctcagtggaacgaaaactcacgttaagggattttggtcatgagattatcaaaaaggatcttcacctagatccttttaaattaaaaatgaagttttaaatcaatctaaagtatatatgagtaaacttggtctgacagttaccaatgcttaatcagtgaggcacctatctcagcgatctgtctatttcgttcatccatagttgcctgactccccgtcgtgtagataactacgatacgggagggcttaccatctggccccagtgctgcaatgataccgcgagacccacgctcaccggctccggatttatcagcaataaaccagccagccggaagggccgagcgcagaagtggtcctgcaactttatccgcctccatccagtctattaattgttgccgggaagctagagtaagtagttcgccagttaatagtttgcgcaacgttgttgccattgctacaggcatcgtggtgtcacgctcgtcgtttggtatggcttcattcagctccggttcccaacgatcaaggcgagttacatgatcccccatgttgtgcaaaaaagcggttagctccttcggtcctccgatcgttgtcagaagtaagttggccgcagtgttatcactcatggttatggcagcactgcataattctcttactgtcatgccatccgtaagatgcttttctgtgactggtgagtactcaaccaagtcattctgagaatagcgtatgcggcgaccgagttgctcttgcccggcgtcaatacgggataataccgcgccacatagcagaactttaaaagtgctcatcattggaaaacgttcttcggggcgaaaactctcaaggatcttaccgctgttgagatccagttcgatgtaacccactcgtgcacccaactgatcttcagcatcttttactttcaccagcgtttctgggtgagcaaaaacaggaaggcaaaatgccgcaaaaaagggaataagggcgacacggaaatgttgaatactcatactcttcctttttcaatattattgaagcatttatcagggttattgtctcatgagcggatacatatttgaatgtatttagaaaaataaacaaataggggttccgcgcacatttccccgaaaagtgccacctgacgtctaagaaaccattattatcatgacattaacctataaaaataggcgtatcacgaggccctttcgtctcgcgcgtttcggtgatgacggtgaaaacctctgacacatgcagctcccggagacggtcacagcttgtctgtaagcggatgccgggagcagacaagcccgtcagggcgcgtcagcgggtgttggcgggtgtcggggctggcttaactatgcggcatcagagcagattgtactgagagtgcaccattcgacgctctcccttatgcgactcctgcattaggaagcagcccagtagtaggttgaggccgttgagcaccgccgccgcaaggaatggtgcatgcaaggagatggcgcccaacagtcccccggccacggggcctgccaccatacccacgccgaaacaagcgctcatgagcccgaagtggcgagcccgatcttccccatcggtgatgtcggcgatataggcgccagcaaccgcacctgtggcgccggtgatgccggccacgatgcgtccggcgtagaggatctggctagcgatgaccctgctgattggttcgctgaccatttccgggtgcgggacggcgttaccagaaactcagaaggttcgtccaaccaaaccgactctggcggcagtttacgagagagatgatagggtctgcttcagtaagccagatgctacacaattaggcttgtacatactgtcgttagaacgcggctacaattaatacataaccttatgtatcatacacatacg

SEQ ID NO: 10 - DNA, 1269 bp, Human coronavirus
atgagcgacaatggaccccagagcaaccagagaagcgcccctaggatcacctttggcggccccaccgattccaccgataacaaccagaatggcggcaggaatggcgctagacccaagcagaggagaccccagggcctgcccaacaataccgcctcctggtttacagctctgacccagcacggaaaggaggagctgagattccccaggggccagggcgtgcctatcaataccaacagcggccccgacgaccagatcggatactacaggagggccaccagaagagtgaggggcggcgacggcaagatgaaagagctgagccccaggtggtacttctactacctgggaaccggccccgaggcttccctgccttatggcgccaacaaggaaggcatcgtgtgggtggccacagaaggcgccctgaacacccccaaggaccacatcggcaccaggaatcccaacaacaacgccgccacagtgctgcagctgccccagggaacaaccctgcccaagggcttttacgccgaaggcagcagaggaggcagccaggctagctccaggagctcctccaggagcaggggcaacagcaggaatagcacccccggatccagcaggggcaatagccctgccaggatggctagcggcggaggagaaaccgccctggctctcctgctgctggacaggctgaatcagttagaaagcaaggtgagcggaaagggccagcagcagcagggccagacagtgaccaagaagtccgctgccgaagcctccaagaagcccaggcagaagagaaccgccaccaagcagtacaacgtgacccaagccttcggcagaaggggccccgaacagacccagggaaacttcggagaccaggatctcatcaggcagggcaccgactacaagcattggcctcagatcgcccagttcgctccctccgcctccgcctttttcggcatgtccagaatcggaatggaggtcacacctagcggcacatggctgacctaccatggcgccattaagctggatgacaaggacccccagttcaaggataacgtgatcctgctgaacaagcacattgacgcctacaagaccttcccccccacagagcctaagaaggataaaaagaaaaagaccgatgaggcccagcccctgccccagagacagaagaagcagcctaccgtgacactgctgcctgccgccgacatggatgacttctccaggcagctgcaaaacagcatgagcggcgcctccgccgatagcacccaggcctga

SEQ ID NO: 11 - DNA, 1242 bp, Human coronavirus
atggctagccccgccgctcctagagccgtgagctttgccgacaacaacgacatcaccaataccaacctgagcaggggcaggggcagaaaccccaagcctagggccgcccccaacaataccgtgagctggtacaccggcctgacccaacacggaaaggtgcccctgacctttccccctggacagggagtgcccctgaacgccaatagcacccccgctcagaatgccggatactggaggagacaggacaggaagatcaataccggcaatggcatcaagcagctggcccccaggtggtacttctattacaccggaaccggacctgaagccgccctgcccttcagagccgtcaaggacggcatcgtgtgggtgcatgaggacggagccacagatgcccccagcaccttcggcaccaggaaccccaacaacgatagcgccatcgtcacccagttcgcccccggaaccaagctgcccaagaacttccacatcgagggcaccggcggaaactcccagtcctcctccagggctagcagcctgtccagaaactccagcaggtcctccagccagggaagcaggagcggcaactccacaagaggcacatcccccggccctagcggcattggcgctgtgggcggagacctgctctacctggatctgctgaatagactgcaggccctggagagcggcaaggtgaagcagagccaacctaaggtcatcaccaagaaggacgccgccgccgctaagaacaagatgagacacaagaggacctccaccaagtccttcaacatggtgcaggccttcggactcagaggacccggcgacctgcagggaaacttcggagacctgcagctgaacaagctgggcacagaggaccccaggtggcctcagatcgccgaactggcccccacagcctccgcctttatgggcatgtcccagttcaagctgacccaccagaacaacgacgatcacggcaaccctgtctacttcctgaggtattccggcgctatcaagctggatcccaagaaccccaactacaacaagtggctggaactgctggagcagaacatcgacgcctacaagaccttccctaagaaggagaaaaagcagaaggcccccaaggaggaaagcaccgatcagatgtccgagccccccaaagagcagagagtgcagggatccattacccagaggacaaggacaagacccagcgtccagcccggccccatgatcgatgtgaacacagactga

SEQ ID NO: 12 - DNA, 1347 bp, Human coronavirus
atgagcttcacacctggcaaacagagcagcagcagagccagcagcggcaacaggagcggcaacggcatcctgaagtgggctgaccaatccgaccagttcagaaacgtgcagacaagaggcagaagggcccagcctaaacagaccgctaccagccaacagccctccggaggcaacgtggtgccctactattcctggttctccggcatcacacagtttcagaagggcaaggagttcgaattcgtggagggccaaggcgtgcccattgctcctggcgtgcctgccacagaggctaagggctactggtacaggcacaacaggaggtccttcaagaccgccgacggcaatcagaggcaactcctgcctaggtggtacttctactacctgggcaccggccctcacgccaaggaccagtatggcaccgacatcgacggcgtgtactgggtcgccagcaaccaggccgacgtgaacacacccgccgacatcgtggacagggaccctagctccgacgaagctatccccaccaggtttcctcctggcaccgtgctgccccagggctactatatcgagggaagcggcaggagcgcccctaacagcagaagcacaagcaggacaagcagcagagccagcagcgccggcagcagatccagggccaatagcggcaataggacacccacctccggcgtgacccccgatatggccgatcagattgcctccctcgtcctggccaagctgggcaaggatgccaccaaaccccagcaggtgaccaaacacaccgccaaggaggtgaggcagaagattctcaacaagcccaggcagaagaggagccccaacaaacagtgcacagtgcagcagtgtttcggcaagaggggccccaaccaaaactttggcggaggcgagatgctgaaactgggaacctccgaccctcaattccccatcctggctgagctggcccctacagccggcgccttcttcttcggaagcagactggagctggccaaggtgcaaaatctgagcggcaatcccgacgagccccagaaggatgtgtacgagctgagatataacggcgccatcaggttcgacagcaccctgtccggcttcgagaccatcatgaaggtgctgaacgagaacctcaacgcctaccagcaacaagacggcatgatgaatatgtcccccaagcctcagagacagaggggccacaagaacggccagggcgagaatgacaacatcagcgtggctgtgcctaaaagcagggtgcagcagaacaagagcagggaactgaccgccgaagacattagcctgctcaaaaagatggatgagccctacaccgaggacaccagcgagatctga

SEQ ID NO: 13 - DNA, 1134 bp, Human coronavirus
atggccagcgtgaattgggccgacgacagggccgctaggaagaagtttcctcccccctccttctacatgcccctgctggtgtccagcgacaaggccccctatagggtgattcccaggaacctggtgcccatcggaaagggcaacaaagacgagcagatcggctactggaacgtgcaggagagatggaggatgagaaggggccagagggtggacctgccccctaaggtgcacttctactatctgggcaccggcccccacaaggacctgaagttcagacagaggtccgacggcgtggtgtgggtggccaaggaaggcgccaagaccgtgaacacctccctgggcaacaggaagaggaaccagaagcccttagaacctaagttcagcatcgccctgcctcctgagctgagcgtcgtcgagttcgaggacagaagcaacaactccagcagggccagcagcaggtccagcaccagaaacaacagcagagattccagcaggtccacatccaggcagcagtccagaacaaggagcgacagcaaccagagcagcagcgatctggtggctgccgtcaccctggccctgaagaacctgggctttgacaaccagagcaagagcccctcctccagcggcaccagcacccctaagaagcctaacaagcccctgagccagcctagggccgacaagcccagccagctcaaaaagcccaggtggaagagggtgcccaccagagaggagaacgtcatccagtgcttcggccccagagacttcaaccacaacatgggcgacagcgacctggtgcagaacggcgtggatgccaagggcttccctcaactggccgaactcatccccaaccaggccgccctgtttttcgacagcgaggtgagcaccgacgaggtgggcgacaacgtgcagatcacctacacctacaagatgctcgtggccaaggacaacaagaacctccccaagttcatcgagcaaatcagcgccttcaccaagcccagcagcatcaaggagatgcagtcccagagctcccacgtggcccagaataccgtgctgaatgccagcattcctgagagcaagcccctggctgacgacgactccgccatcatcgagatcgtgaacgaggtgctgcactga

SEQ ID NO: 14 - DNA, 1326 bp, Human coronavirus
atgtcctacacacccggccactacgccggcagcagatccagcagcggcaacagatccggcatcctgaaaaagaccagctgggctgaccaatccgagaggaactaccagaccttcaacaggggaaggaaaacccagcccaaattcaccgtgagcacacagcctcagggcaacaccatcccccactacagctggttcagcggcatcacccaattccagaagggcagggactttaagttctccgacggccagggcgtgcctattgccttcggcgtccctcccagcgaagctaagggctattggtacaggcactccaggaggtcctttaagacagccgacggccagcagaagcagctgctgcctaggtggtacttctattacctgggcaccggcccctacgccaatgctagctacggcgagagcctggagggcgtgttctgggtggccaaccaccaagccgacaccagcacccccagcgatgtctccagcagggatcctaccacccaggaggccatccccaccagattccctcccggaacaattctgccccagggctactatgtggagggcagcggcaggagcgctagcaactccagacccggatccagatcccagtccagaggccccaacaacaggtccctgtccaggagcaactccaacttcaggcacagcgacagcatcgtgaaacccgacatggccgatgagattgccaacctggtgctggccaagctcggcaaagactccaaaccccagcaagtgaccaagcagaacgccaaggagatcaggcataagatcctgaccaagcccaggcagaagaggacccctaacaagcactgcaacgtgcagcagtgcttcggcaagagaggccccagccagaacttcggaaacgccgaaatgctgaagctgggcaccaatgatccccagtttcccatcctcgccgaactggcccccacccccggcgctttcttttttggcagcaagctggacctggtgaagagggatagcgaggccgattcccccgtgaaggatgtgttcgagctgcactacagcggctccatcagattcgactccaccctgcccggcttcgagaccatcatgaaggtcttagaagagaacctgaatgcctacgtgaacagcaaccagaataccgacagcgacagcctgagctccaagccccagaggaagaggggcgtcaagcagctgcccgagcagttcgacagcctgaatctgagcgctggcacacagcacatcagcaatgacttcacacccgaagaccacagcctcctggccacactcgacgatccctatgtggaagatagcgtggcctga

SEQ ID NO: 15 - DNA, 1170 bp, Human coronavirus
atggccaccgtgaagtgggctgacgcttccgagcctcagaggggcagacagggcaggatcccctatagcctgtactcccctctgctggtggacagcgagcagccctggaaggtgatccctaggaatctggtgcccatcaacaagaaggataagaacaagctcatcggctactggaacgtccaaaagagattcaggaccagaaagggcaagagagtcgacctcagccctaagctgcacttctactacctgggcaccggcccccacaaagacgccaaattcagagagagggtggagggcgtggtgtgggtcgctgtggatggcgccaagacagaacccaccggctacggcgtgagaagaaagaactccgagcccgagattccccactttaaccagaaactgcccaacggagtgaccgtggtggaggagcctgatagcagggcccctagcaggagccagagcaggagccaaagcaggggcaggggcgaaagcaagccccagagcaggaatcccagctccgacagaaaccataactcccaggacgacatcatgaaggccgtggctgccgccctgaagagcctgggcttcgacaagccccaggagaaggacaagaagagcgctaagaccggcacacccaagccttccaggaaccagtcccccgcctcctcccaaaccagcgccaagagcctcgccaggagccaatccagcgagaccaaggagcagaagcacgagatgcagaagcccaggtggaagaggcagcctaatgacgatgtgaccagcaacgtgacccagtgcttcggccccagggacctggatcacaacttcggctccgctggcgtcgtcgccaatggcgtgaaagccaagggatacccccagttcgccgaactggtcccttccacagctgccatgctgttcgacagccacatcgtgtccaaggagtccggaaataccgtggtgctgaccttcaccacaagggtgaccgtgcctaaggaccaccctcacctgggcaagttcctggaggagctcaacgcctttaccagggagatgcagcagcaccccctgctgaacccttccgccctggagttcaatccctcccagacaagccccgccacagctgagcctgtgagggacgaggtgagcatcgagaccgatatcatcgatgaggtgaattga